European Patent Application EP 4 636 096 A2, published October 22, 2025. Title: SYNTHESIZING BARCODING SEQUENCES UTILIZING PHASE-SHIFT BLOCKS AND USES THEREOF. Applicant: Bio-Rad Laboratories, Inc. Application EP EP17738940.0, filed January 12, 2017. The sequence listing filed with the application follows.

SEQUENCE LISTING (118 sequences)

SEQ ID NO: 1 - DNA, 62 bp, synthetic construct
  misc_feature 1..62: note = synthetic polynucleotide
  misc_feature 15..20: note = n = any nucleotide
  misc_feature 36..41: note = n = any nucleotide
  misc_feature 57..62: note = n = any nucleotide
  source 1..62: mol_type = other DNA
cgctcttccgatctnnnnnngtgcgctgatcggagnnnnnntcggcatgtctggctnnnnnn

SEQ ID NO: 2 - DNA, 63 bp, synthetic construct
  misc_feature 1..63: note = synthetic polynucleotide
  misc_feature 16..21: note = n = any nucleotide
  misc_feature 37..42: note = n = any nucleotide
  misc_feature 58..63: note = n = any nucleotide
  source 1..63: mol_type = other DNA
cgctcttccgatctannnnnngtgcgctgatcggagnnnnnntcggcatgtctggctnnnnnn

SEQ ID NO: 3 - DNA, 64 bp, synthetic construct
  misc_feature 1..64: note = synthetic polynucleotide
  misc_feature 17..22: note = n = any nucleotide
  misc_feature 38..43: note = n = any nucleotide
  misc_feature 59..64: note = n = any nucleotide
  source 1..64: mol_type = other DNA
cgctcttccgatctcannnnnngtgcgctgatcggagnnnnnntcggcatgtctggctnnnnnn

SEQ ID NO: 4 - DNA, 65 bp, synthetic construct
  misc_feature 1..65: note = synthetic polynucleotide
  misc_feature 18..23: note = n = any nucleotide
  misc_feature 39..44: note = n = any nucleotide
  misc_feature 60..65: note = n = any nucleotide
  source 1..65: mol_type = other DNA
cgctcttccgatctgcannnnnngtgcgctgatcggagnnnnnntcggcatgtctggctnnnnnn

SEQ ID NO: 5 - DNA, 66 bp, synthetic construct
  misc_feature 1..66: note = synthetic polynucleotide
  misc_feature 19..24: note = n = any nucleotide
  misc_feature 40..45: note = n = any nucleotide
  misc_feature 61..66: note = n = any nucleotide
  source 1..66: mol_type = other DNA
cgctcttccgatcttgcannnnnngtgcgctgatcggagnnnnnntcggcatgtctggctnnnnnn

SEQ ID NO: 6 - DNA, 16 bp, synthetic construct
  misc_feature 1..16: note = synthetic oligonucleotide
  source 1..16: mol_type = other DNA
cgtactctgcgttgat

SEQ ID NO: 7 - DNA, 15 bp, synthetic construct
  misc_feature 1..15: note = synthetic oligonucleotide
  source 1..15: mol_type = other DNA
gcaatgcgatggcta

SEQ ID NO: 8 - DNA, 15 bp, synthetic construct
  misc_feature 1..15: note = synthetic oligonucleotide
  source 1..15: mol_type = other DNA
ttcagctcagtggta

SEQ ID NO: 9 - skipped

SEQ ID NO: 10 - DNA, 21 bp, synthetic construct
  misc_feature 1..21: note = synthetic oligonucleotide
  source 1..21: mol_type = other DNA
baaaaaaaaaaaaaaaaaaaa

SEQ ID NO: 11 - DNA, 54 bp, synthetic construct
  misc_feature 1..54: note = synthetic polynucleotide
  source 1..54: mol_type = other DNA
ttttttttttctacacgcctgtccgcggaagcagtggtatcaacgcagagtacg

SEQ ID NO: 12 - DNA, 38 bp, synthetic construct
  misc_feature 1..38: note = synthetic polynucleotide
  misc_feature 16..21: note = n = any nucleotide
  source 1..38: mol_type = other DNA
gcaatgcgatggctannnnnnacgtactctgcgttgat

SEQ ID NO: 13 - DNA, 39 bp, synthetic construct
  misc_feature 1..39: note = synthetic polynucleotide
  misc_feature 16..21: note = n = any nucleotide
  source 1..39: mol_type = other DNA
gcaatgcgatggctannnnnnaccgtactctgcgttgat

SEQ ID NO: 14 - DNA, 40 bp, synthetic construct
  misc_feature 1..40: note = synthetic polynucleotide
  misc_feature 16..21: note = n = any nucleotide
  source 1..40: mol_type = other DNA
gcaatgcgatggctannnnnnacgcgtactctgcgttgat

SEQ ID NO: 15 - DNA, 41 bp, synthetic construct
  misc_feature 1..41: note = synthetic polynucleotide
  misc_feature 16..21: note = n = any nucleotide
  source 1..41: mol_type = other DNA
gcaatgcgatggctannnnnnacgtcgtactctgcgttgat

SEQ ID NO: 16 - DNA, 76 bp, synthetic construct
  misc_feature 1..76: note = synthetic polynucleotide
  misc_feature 56..61: note = n = any nucleotide
  source 1..76: mol_type = other DNA
ttttttttttctacacgcctgtccgcggaagcagtggtatcaacgcagagtacgtnnnnnntagccatcgcattgc

SEQ ID NO: 17 - DNA, 48 bp, synthetic construct
  misc_feature 1..48: note = synthetic polynucleotide
  misc_feature 16..21: note = n = any nucleotide
  source 1..48: mol_type = other DNA
gcaatgcgatggctannnnnnacgtactctgcgttgataccactgctt

SEQ ID NO: 18 - DNA, 36 bp, synthetic construct
  misc_feature 1..36: note = synthetic polynucleotide
  misc_feature 16..21: note = n = any nucleotide
  source 1..36: mol_type = other DNA
ttcagctcagtggtannnnnngcaatgcgatggcta

SEQ ID NO: 19 - DNA, 97 bp, synthetic construct
  misc_feature 1..97: note = synthetic polynucleotide
  misc_feature 56..61: note = n = any nucleotide
  misc_feature 77..82: note = n = any nucleotide
  source 1..97: mol_type = other DNA
ttttttttttctacacgcctgtccgcggaagcagtggtatcaacgcagagtacgtnnnnnntagccatcgcattgcnnnnnntaccactgagctgaa

SEQ ID NO: 20 - DNA, 53 bp, synthetic construct
  misc_feature 1..53: note = synthetic polynucleotide
  misc_feature 22..29: note = n = any nucleotide
  misc_feature 33..38: note = n = any nucleotide
  source 1..53: mol_type = other DNA
baaaaaaaaaaaaaaaaaaaannnnnnnncgtnnnnnnttcagctcagtggta

SEQ ID NO: 21 - DNA, 95 bp, synthetic construct
  misc_feature 1..95: note = synthetic polynucleotide
  misc_feature 13..18: note = n = any nucleotide
  misc_feature 34..39: note = n = any nucleotide
  misc_feature 55..60: note = n = any nucleotide
  misc_feature 64..71: note = n = any nucleotide
  source 1..95: mol_type = other DNA
cgcagagtacgtnnnnnntagccatcgcattgcnnnnnntaccactgagctgaannnnnnacgnnnnnnnnacgttttttttttttttttttttv

SEQ ID NO: 22 - DNA, 144 bp, synthetic construct
  misc_feature 1..144: note = synthetic polynucleotide
  misc_feature 55: note = n = a
  misc_feature 56: note = n = c or absent
  misc_feature 57: note = n =g or absent if nucleotide in position 56 is absent
  misc_feature 58: note = n= t or absent if nucleotides in position 56 and 57 are absent
  misc_feature 60..65: note = n = any nucleotide
  misc_feature 81..86: note = n = any nucleotide
  misc_feature 102..109: note = n = any nucleotide
  misc_feature 113..120: note = n = any nucleotide
  source 1..144: mol_type = other DNA
ttttttttttctacacgcctgtccgcggaagcagtggtatcaacgcagagtacgnnnntnnnnnntagccatcgcattgcnnnnnntaccactgagctgaannnnnnnnacgnnnnnnnntgcaaaaaaaaaaaaaaaaaaaab

SEQ ID NO: 23 - DNA, 37 bp, synthetic construct
  misc_feature 1..37: note = synthetic polynucleotide
  misc_feature 17..22: note = n = any nucleotide
  source 1..37: mol_type = other DNA
tagttgcgtctcatgcnnnnnnatcggtagcgtaacg

SEQ ID NO: 24 - DNA, 37 bp, synthetic construct; identical to SEQ ID NO: 23
  misc_feature 1..37: note = synthetic polynucleotide
  misc_feature 17..22: note = n = any nucleotide
  source 1..37: mol_type = other DNA

SEQ ID NO: 25 - DNA, 37 bp, synthetic construct; identical to SEQ ID NO: 23
  misc_feature 1..37: note = synthetic polynucleotide
  misc_feature 17..22: note = n = any nucleotide
  source 1..37: mol_type = other DNA

SEQ ID NO: 26 - DNA, 37 bp, synthetic construct
  misc_feature 1..37: note = synthetic polynucleotide
  misc_feature 17..22: note = n = any nucleotide
  source 1..37: mol_type = other DNA
tagttgcgtctcatgcnnnnnngcatgcgttactgga

SEQ ID NO: 27 - DNA, 37 bp, synthetic construct; identical to SEQ ID NO: 26
  misc_feature 1..37: note = synthetic polynucleotide
  misc_feature 17..22: note = n = any nucleotide
  source 1..37: mol_type = other DNA

SEQ ID NO: 28 - DNA, 37 bp, synthetic construct; identical to SEQ ID NO: 26
  misc_feature 1..37: note = synthetic polynucleotide
  misc_feature 17..22: note = n = any nucleotide
  source 1..37: mol_type = other DNA

SEQ ID NO: 29 - DNA, 37 bp, synthetic construct
  misc_feature 1..37: note = synthetic polynucleotide
  misc_feature 17..22: note = n = any nucleotide
  source 1..37: mol_type = other DNA
tagttgcgtctcatgcnnnnnncgtatagcgtagttc

SEQ ID NO: 30 - DNA, 37 bp, synthetic construct; identical to SEQ ID NO: 29
  misc_feature 1..37: note = synthetic polynucleotide
  misc_feature 17..22: note = n = any nucleotide
  source 1..37: mol_type = other DNA

SEQ ID NO: 31 - DNA, 37 bp, synthetic construct; identical to SEQ ID NO: 29
  misc_feature 1..37: note = synthetic polynucleotide
  misc_feature 17..22: note = n = any nucleotide
  source 1..37: mol_type = other DNA

SEQ ID NO: 32 - DNA, 36 bp, synthetic construct
  misc_feature 1..36: note = synthetic polynucleotide
  misc_feature 16..21: note = n = any nucleotide
  source 1..36: mol_type = other DNA
tagccatcgcattgcnnnnnnttactggcactgatc

SEQ ID NO: 33 - DNA, 36 bp, synthetic construct; identical to SEQ ID NO: 32
  misc_feature 1..36: note = synthetic polynucleotide
  misc_feature 16..21: note = n = any nucleotide
  source 1..36: mol_type = other DNA

SEQ ID NO: 34 - DNA, 36 bp, synthetic construct; identical to SEQ ID NO: 32
  misc_feature 1..36: note = synthetic polynucleotide
  misc_feature 16..21: note = n = any nucleotide
  source 1..36: mol_type = other DNA

SEQ ID NO: 35 - DNA, 36 bp, synthetic construct; identical to SEQ ID NO: 32
  misc_feature 1..36: note = synthetic polynucleotide
  misc_feature 16..21: note = n = any nucleotide
  source 1..36: mol_type = other DNA

SEQ ID NO: 36 - DNA, 36 bp, synthetic construct; identical to SEQ ID NO: 32
  misc_feature 1..36: note = synthetic polynucleotide
  misc_feature 16..21: note = n = any nucleotide
  source 1..36: mol_type = other DNA

SEQ ID NO: 37 - DNA, 36 bp, synthetic construct; identical to SEQ ID NO: 32
  misc_feature 1..36: note = synthetic polynucleotide
  misc_feature 16..21: note = n = any nucleotide
  source 1..36: mol_type = other DNA

SEQ ID NO: 38 - DNA, 36 bp, synthetic construct; identical to SEQ ID NO: 32
  misc_feature 1..36: note = synthetic polynucleotide
  misc_feature 16..21: note = n = any nucleotide
  source 1..36: mol_type = other DNA

SEQ ID NO: 39 - DNA, 36 bp, synthetic construct; identical to SEQ ID NO: 32
  misc_feature 1..36: note = synthetic polynucleotide
  misc_feature 16..21: note = n = any nucleotide
  source 1..36: mol_type = other DNA

SEQ ID NO: 40 - DNA, 36 bp, synthetic construct; identical to SEQ ID NO: 32
  misc_feature 1..36: note = synthetic polynucleotide
  misc_feature 16..21: note = n = any nucleotide
  source 1..36: mol_type = other DNA

SEQ ID NO: 41 - DNA, 36 bp, synthetic construct
  misc_feature 1..36: note = synthetic polynucleotide
  misc_feature 16..21: note = n = any nucleotide
  source 1..36: mol_type = other DNA
cgtacgcaatgacctnnnnnngcgcatttatgccat

SEQ ID NO: 42 - DNA, 36 bp, synthetic construct; identical to SEQ ID NO: 41
  misc_feature 1..36: note = synthetic polynucleotide
  misc_feature 16..21: note = n = any nucleotide
  source 1..36: mol_type = other DNA

SEQ ID NO: 43 - DNA, 36 bp, synthetic construct; identical to SEQ ID NO: 41
  misc_feature 1..36: note = synthetic polynucleotide
  misc_feature 16..21: note = n = any nucleotide
  source 1..36: mol_type = other DNA

SEQ ID NO: 44 - DNA, 36 bp, synthetic construct; identical to SEQ ID NO: 41
  misc_feature 1..36: note = synthetic polynucleotide
  misc_feature 16..21: note = n = any nucleotide
  source 1..36: mol_type = other DNA

SEQ ID NO: 45 - DNA, 36 bp, synthetic construct; identical to SEQ ID NO: 41
  misc_feature 1..36: note = synthetic polynucleotide
  misc_feature 16..21: note = n = any nucleotide
  source 1..36: mol_type = other DNA

SEQ ID NO: 46 - DNA, 36 bp, synthetic construct; identical to SEQ ID NO: 41
  misc_feature 1..36: note = synthetic polynucleotide
  misc_feature 16..21: note = n = any nucleotide
  source 1..36: mol_type = other DNA

SEQ ID NO: 47 - DNA, 36 bp, synthetic construct; identical to SEQ ID NO: 41
  misc_feature 1..36: note = synthetic polynucleotide
  misc_feature 16..21: note = n = any nucleotide
  source 1..36: mol_type = other DNA

SEQ ID NO: 48 - DNA, 36 bp, synthetic construct; identical to SEQ ID NO: 41
  misc_feature 1..36: note = synthetic polynucleotide
  misc_feature 16..21: note = n = any nucleotide
  source 1..36: mol_type = other DNA

SEQ ID NO: 49 - DNA, 36 bp, synthetic construct; identical to SEQ ID NO: 41
  misc_feature 1..36: note = synthetic polynucleotide
  misc_feature 16..21: note = n = any nucleotide
  source 1..36: mol_type = other DNA

SEQ ID NO: 50 - DNA, 36 bp, synthetic construct
  misc_feature 1..36: note = synthetic polynucleotide
  misc_feature 16..21: note = n = any nucleotide
  source 1..36: mol_type = other DNA
gcatatcgcatcaagnnnnnncatggatcggtcatg

SEQ ID NO: 51 - DNA, 36 bp, synthetic construct; identical to SEQ ID NO: 50
  misc_feature 1..36: note = synthetic polynucleotide
  misc_feature 16..21: note = n = any nucleotide
  source 1..36: mol_type = other DNA

SEQ ID NO: 52 - DNA, 36 bp, synthetic construct; identical to SEQ ID NO: 50
  misc_feature 1..36: note = synthetic polynucleotide
  misc_feature 16..21: note = n = any nucleotide
  source 1..36: mol_type = other DNA

SEQ ID NO: 53 - DNA, 36 bp, synthetic construct; identical to SEQ ID NO: 50
  misc_feature 1..36: note = synthetic polynucleotide
  misc_feature 16..21: note = n = any nucleotide
  source 1..36: mol_type = other DNA

SEQ ID NO: 54 - DNA, 36 bp, synthetic construct; identical to SEQ ID NO: 50
  misc_feature 1..36: note = synthetic polynucleotide
  misc_feature 16..21: note = n = any nucleotide
  source 1..36: mol_type = other DNA

SEQ ID NO: 55 - DNA, 36 bp, synthetic construct; identical to SEQ ID NO: 50
  misc_feature 1..36: note = synthetic polynucleotide
  misc_feature 16..21: note = n = any nucleotide
  source 1..36: mol_type = other DNA

SEQ ID NO: 56 - DNA, 36 bp, synthetic construct; identical to SEQ ID NO: 50
  misc_feature 1..36: note = synthetic polynucleotide
  misc_feature 16..21: note = n = any nucleotide
  source 1..36: mol_type = other DNA

SEQ ID NO: 57 - DNA, 36 bp, synthetic construct; identical to SEQ ID NO: 50
  misc_feature 1..36: note = synthetic polynucleotide
  misc_feature 16..21: note = n = any nucleotide
  source 1..36: mol_type = other DNA

SEQ ID NO: 58 - DNA, 36 bp, synthetic construct; identical to SEQ ID NO: 50
  misc_feature 1..36: note = synthetic polynucleotide
  misc_feature 16..21: note = n = any nucleotide
  source 1..36: mol_type = other DNA

SEQ ID NO: 59 - DNA, 36 bp, synthetic construct
  misc_feature 1..36: note = synthetic polynucleotide
  misc_feature 16..27: note = n = any nucleotide
  source 1..36: mol_type = other DNA
aatgaccgtgactatnnnnnnnnnnnnttttttttt

SEQ ID NO: 60 - DNA, 36 bp, synthetic construct; identical to SEQ ID NO: 59
  misc_feature 1..36: note = synthetic polynucleotide
  misc_feature 16..27: note = n = any nucleotide
  source 1..36: mol_type = other DNA

SEQ ID NO: 61 - DNA, 36 bp, synthetic construct; identical to SEQ ID NO: 59
  misc_feature 1..36: note = synthetic polynucleotide
  misc_feature 16..27: note = n = any nucleotide
  source 1..36: mol_type = other DNA

SEQ ID NO: 62 - DNA, 36 bp, synthetic construct; identical to SEQ ID NO: 59
  misc_feature 1..36: note = synthetic polynucleotide
  misc_feature 16..27: note = n = any nucleotide
  source 1..36: mol_type = other DNA

SEQ ID NO: 63 - DNA, 36 bp, synthetic construct; identical to SEQ ID NO: 59
  misc_feature 1..36: note = synthetic polynucleotide
  misc_feature 16..27: note = n = any nucleotide
  source 1..36: mol_type = other DNA

SEQ ID NO: 64 - DNA, 36 bp, synthetic construct; identical to SEQ ID NO: 59
  misc_feature 1..36: note = synthetic polynucleotide
  misc_feature 16..27: note = n = any nucleotide
  source 1..36: mol_type = other DNA

SEQ ID NO: 65 - DNA, 36 bp, synthetic construct; identical to SEQ ID NO: 59
  misc_feature 1..36: note = synthetic polynucleotide
  misc_feature 16..27: note = n = any nucleotide
  source 1..36: mol_type = other DNA

SEQ ID NO: 66 - DNA, 36 bp, synthetic construct; identical to SEQ ID NO: 59
  misc_feature 1..36: note = synthetic polynucleotide
  misc_feature 16..27: note = n = any nucleotide
  source 1..36: mol_type = other DNA

SEQ ID NO: 67 - DNA, 36 bp, synthetic construct; identical to SEQ ID NO: 59
  misc_feature 1..36: note = synthetic polynucleotide
  misc_feature 16..27: note = n = any nucleotide
  source 1..36: mol_type = other DNA

SEQ ID NO: 68 - DNA, 36 bp, synthetic construct
  misc_feature 1..36: note = synthetic polynucleotide
  misc_feature 16..27: note = n = any nucleotide
  source 1..36: mol_type = other DNA
cgcgtaaatacggtannnnnnnnnnnnttttttttt

SEQ ID NO: 69 - DNA, 36 bp, synthetic construct; identical to SEQ ID NO: 68
  misc_feature 1..36: note = synthetic polynucleotide
  misc_feature 16..27: note = n = any nucleotide
  source 1..36: mol_type = other DNA

SEQ ID NO: 70 - DNA, 36 bp, synthetic construct; identical to SEQ ID NO: 68
  misc_feature 1..36: note = synthetic polynucleotide
  misc_feature 16..27: note = n = any nucleotide
  source 1..36: mol_type = other DNA

SEQ ID NO: 71 - DNA, 36 bp, synthetic construct; identical to SEQ ID NO: 68
  misc_feature 1..36: note = synthetic polynucleotide
  misc_feature 16..27: note = n = any nucleotide
  source 1..36: mol_type = other DNA

SEQ ID NO: 72 - DNA, 36 bp, synthetic construct; identical to SEQ ID NO: 68
  misc_feature 1..36: note = synthetic polynucleotide
  misc_feature 16..27: note = n = any nucleotide
  source 1..36: mol_type = other DNA

SEQ ID NO: 73 - DNA, 36 bp, synthetic construct; identical to SEQ ID NO: 68
  misc_feature 1..36: note = synthetic polynucleotide
  misc_feature 16..27: note = n = any nucleotide
  source 1..36: mol_type = other DNA

SEQ ID NO: 74 - DNA, 36 bp, synthetic construct; identical to SEQ ID NO: 68
  misc_feature 1..36: note = synthetic polynucleotide
  misc_feature 16..27: note = n = any nucleotide
  source 1..36: mol_type = other DNA

SEQ ID NO: 75 - DNA, 36 bp, synthetic construct; identical to SEQ ID NO: 68
  misc_feature 1..36: note = synthetic polynucleotide
  misc_feature 16..27: note = n = any nucleotide
  source 1..36: mol_type = other DNA

SEQ ID NO: 76 - DNA, 36 bp, synthetic construct; identical to SEQ ID NO: 68
  misc_feature 1..36: note = synthetic polynucleotide
  misc_feature 16..27: note = n = any nucleotide
  source 1..36: mol_type = other DNA

SEQ ID NO: 77 - DNA, 36 bp, synthetic construct
  misc_feature 1..36: note = synthetic polynucleotide
  misc_feature 16..27: note = n = any nucleotide
  source 1..36: mol_type = other DNA
gtacctagccagtacnnnnnnnnnnnnttttttttt

SEQ ID NO: 78 - DNA, 36 bp, synthetic construct; identical to SEQ ID NO: 77
  misc_feature 1..36: note = synthetic polynucleotide
  misc_feature 16..27: note = n = any nucleotide
  source 1..36: mol_type = other DNA

SEQ ID NO: 79 - DNA, 36 bp, synthetic construct; identical to SEQ ID NO: 77
  misc_feature 1..36: note = synthetic polynucleotide
  misc_feature 16..27: note = n = any nucleotide
  source 1..36: mol_type = other DNA

SEQ ID NO: 80 - DNA, 36 bp, synthetic construct; identical to SEQ ID NO: 77
  misc_feature 1..36: note = synthetic polynucleotide
  misc_feature 16..27: note = n = any nucleotide
  source 1..36: mol_type = other DNA

SEQ ID NO: 81 - DNA, 36 bp, synthetic construct; identical to SEQ ID NO: 77
  misc_feature 1..36: note = synthetic polynucleotide
  misc_feature 16..27: note = n = any nucleotide
  source 1..36: mol_type = other DNA

SEQ ID NO: 82 - DNA, 36 bp, synthetic construct; identical to SEQ ID NO: 77
  misc_feature 1..36: note = synthetic polynucleotide
  misc_feature 16..27: note = n = any nucleotide
  source 1..36: mol_type = other DNA

SEQ ID NO: 83 - DNA, 36 bp, synthetic construct; identical to SEQ ID NO: 77
  misc_feature 1..36: note = synthetic polynucleotide
  misc_feature 16..27: note = n = any nucleotide
  source 1..36: mol_type = other DNA

SEQ ID NO: 84 - DNA, 36 bp, synthetic construct; identical to SEQ ID NO: 77
  misc_feature 1..36: note = synthetic polynucleotide
  misc_feature 16..27: note = n = any nucleotide
  source 1..36: mol_type = other DNA

SEQ ID NO: 85 - DNA, 36 bp, synthetic construct; identical to SEQ ID NO: 77
  misc_feature 1..36: note = synthetic polynucleotide
  misc_feature 16..27: note = n = any nucleotide
  source 1..36: mol_type = other DNA

SEQ ID NO: 86 - DNA, 79 bp, synthetic construct
  misc_feature 1..79: note = synthetic polynucleotide
  misc_feature 17..22: note = n = any nucleotide
  misc_feature 38..43: note = n = any nucleotide
  misc_feature 59..70: note = n = any nucleotide
  source 1..79: mol_type = other DNA
tagttgcgtctcatgcnnnnnnatcgatagcgtaacgnnnnnnttactggcactgatcnnnnnnnnnnnnttttttttt

SEQ ID NO: 87 - DNA, 79 bp, synthetic construct; identical to SEQ ID NO: 86
  misc_feature 1..79: note = synthetic polynucleotide
  misc_feature 17..22: note = n = any nucleotide
  misc_feature 38..43: note = n = any nucleotide
  misc_feature 59..70: note = n = any nucleotide
  source 1..79: mol_type = other DNA

SEQ ID NO: 88 - DNA, 37 bp, synthetic construct
  misc_feature 1..37: note = synthetic polynucleotide
  misc_feature 17..22: note = n = any nucleotide
  source 1..37: mol_type = other DNA
tagttgcgtctcatgcnnnnnnatcgatagcgtaacg

SEQ ID NO: 89 - DNA, 37 bp, synthetic construct; identical to SEQ ID NO: 88
  misc_feature 1..37: note = synthetic polynucleotide
  misc_feature 17..22: note = n = any nucleotide
  source 1..37: mol_type = other DNA

SEQ ID NO: 90 - DNA, 37 bp, synthetic construct; identical to SEQ ID NO: 88
  misc_feature 1..37: note = synthetic polynucleotide
  misc_feature 17..22: note = n = any nucleotide
  source 1..37: mol_type = other DNA

SEQ ID NO: 91 - DNA, 37 bp, synthetic construct; identical to SEQ ID NO: 88
  misc_feature 1..37: note = synthetic polynucleotide
  misc_feature 17..22: note = n = any nucleotide
  source 1..37: mol_type = other DNA

SEQ ID NO: 92 - DNA, 38 bp, synthetic construct
  misc_feature 1..38: note = synthetic polynucleotide
  misc_feature 17..22: note = n = any nucleotide
  source 1..38: mol_type = other DNA
tagttgcgtctcatgcnnnnnngatcgatagcgtaacg

SEQ ID NO: 93 - DNA, 38 bp, synthetic construct; identical to SEQ ID NO: 92
  misc_feature 1..38: note = synthetic polynucleotide
  misc_feature 17..22: note = n = any nucleotide
  source 1..38: mol_type = other DNA

SEQ ID NO: 94 - DNA, 39 bp, synthetic construct
  misc_feature 1..39: note = synthetic polynucleotide
  misc_feature 17..22: note = n = any nucleotide
  source 1..39: mol_type = other DNA
tagttgcgtctcatgcnnnnnngcatcgatagcgtaacg

SEQ ID NO: 95 - DNA, 39 bp, synthetic construct; identical to SEQ ID NO: 94
  misc_feature 1..39: note = synthetic polynucleotide
  misc_feature 17..22: note = n = any nucleotide
  source 1..39: mol_type = other DNA

SEQ ID NO: 96 - DNA, 39 bp, synthetic construct; identical to SEQ ID NO: 94
  misc_feature 1..39: note = synthetic polynucleotide
  misc_feature 17..22: note = n = any nucleotide
  source 1..39: mol_type = other DNA

SEQ ID NO: 97 - DNA, 36 bp, synthetic construct; identical to SEQ ID NO: 32
  misc_feature 1..36: note = synthetic polynucleotide
  misc_feature 16..21: note = n = any nucleotide
  source 1..36: mol_type = other DNA

SEQ ID NO: 98 - DNA, 36 bp, synthetic construct; identical to SEQ ID NO: 32
  misc_feature 1..36: note = synthetic polynucleotide
  misc_feature 16..21: note = n = any nucleotide
  source 1..36: mol_type = other DNA

SEQ ID NO: 99 - DNA, 36 bp, synthetic construct; identical to SEQ ID NO: 32
  misc_feature 1..36: note = synthetic polynucleotide
  misc_feature 16..21: note = n = any nucleotide
  source 1..36: mol_type = other DNA

SEQ ID NO: 100 - DNA, 36 bp, synthetic construct; identical to SEQ ID NO: 32
  misc_feature 1..36: note = synthetic polynucleotide
  misc_feature 16..21: note = n = any nucleotide
  source 1..36: mol_type = other DNA

SEQ ID NO: 101 - DNA, 36 bp, synthetic construct; identical to SEQ ID NO: 32
  misc_feature 1..36: note = synthetic polynucleotide
  misc_feature 16..21: note = n = any nucleotide
  source 1..36: mol_type = other DNA

SEQ ID NO: 102 - DNA, 36 bp, synthetic construct; identical to SEQ ID NO: 32
  misc_feature 1..36: note = synthetic polynucleotide
  misc_feature 16..21: note = n = any nucleotide
  source 1..36: mol_type = other DNA

SEQ ID NO: 103 - DNA, 36 bp, synthetic construct; identical to SEQ ID NO: 32
  misc_feature 1..36: note = synthetic polynucleotide
  misc_feature 16..21: note = n = any nucleotide
  source 1..36: mol_type = other DNA

SEQ ID NO: 104 - DNA, 36 bp, synthetic construct; identical to SEQ ID NO: 32
  misc_feature 1..36: note = synthetic polynucleotide
  misc_feature 16..21: note = n = any nucleotide
  source 1..36: mol_type = other DNA

SEQ ID NO: 105 - DNA, 36 bp, synthetic construct; identical to SEQ ID NO: 32
  misc_feature 1..36: note = synthetic polynucleotide
  misc_feature 16..21: note = n = any nucleotide
  source 1..36: mol_type = other DNA

SEQ ID NO: 106 - DNA, 36 bp, synthetic construct
  misc_feature 1..36: note = synthetic polynucleotide
  misc_feature 16..27: note = n = any nucleotide
  source 1..36: mol_type = other DNA
aatgaccgtgactagnnnnnnnnnnnnttttttttt

SEQ ID NO: 107 - DNA, 36 bp, synthetic construct; identical to SEQ ID NO: 106
  misc_feature 1..36: note = synthetic polynucleotide
  misc_feature 16..27: note = n = any nucleotide
  source 1..36: mol_type = other DNA

SEQ ID NO: 108 - DNA, 36 bp, synthetic construct; identical to SEQ ID NO: 106
  misc_feature 1..36: note = synthetic polynucleotide
  misc_feature 16..27: note = n = any nucleotide
  source 1..36: mol_type = other DNA

SEQ ID NO: 109 - DNA, 36 bp, synthetic construct; identical to SEQ ID NO: 106
  misc_feature 1..36: note = synthetic polynucleotide
  misc_feature 16..27: note = n = any nucleotide
  source 1..36: mol_type = other DNA

SEQ ID NO: 110 - DNA, 36 bp, synthetic construct; identical to SEQ ID NO: 106
  misc_feature 1..36: note = synthetic polynucleotide
  misc_feature 16..27: note = n = any nucleotide
  source 1..36: mol_type = other DNA

SEQ ID NO: 111 - DNA, 36 bp, synthetic construct; identical to SEQ ID NO: 106
  misc_feature 1..36: note = synthetic polynucleotide
  misc_feature 16..27: note = n = any nucleotide
  source 1..36: mol_type = other DNA

SEQ ID NO: 112 - DNA, 36 bp, synthetic construct; identical to SEQ ID NO: 106
  misc_feature 1..36: note = synthetic polynucleotide
  misc_feature 16..27: note = n = any nucleotide
  source 1..36: mol_type = other DNA

SEQ ID NO: 113 - DNA, 36 bp, synthetic construct; identical to SEQ ID NO: 106
  misc_feature 1..36: note = synthetic polynucleotide
  misc_feature 16..27: note = n = any nucleotide
  source 1..36: mol_type = other DNA

SEQ ID NO: 114 - DNA, 36 bp, synthetic construct; identical to SEQ ID NO: 106
  misc_feature 1..36: note = synthetic polynucleotide
  misc_feature 16..27: note = n = any nucleotide
  source 1..36: mol_type = other DNA

SEQ ID NO: 115 - DNA, 79 bp, synthetic construct; identical to SEQ ID NO: 86
  misc_feature 1..79: note = synthetic polynucleotide
  misc_feature 17..22: note = n = any nucleotide
  misc_feature 38..43: note = n = any nucleotide
  misc_feature 59..70: note = n = any nucleotide
  source 1..79: mol_type = other DNA

SEQ ID NO: 116 - DNA, 81 bp, synthetic construct
  misc_feature 1..81: note = synthetic polynucleotide
  misc_feature 17..22: note = n = any nucleotide
  misc_feature 40..45: note = n = any nucleotide
  misc_feature 61..72: note = n = any nucleotide
  source 1..81: mol_type = other DNA
tagttgcgtctcatgcnnnnnngcatcgatagcgtaacgnnnnnnttactggcactgatcnnnnnnnnnnnnttttttttt

SEQ ID NO: 117 - DNA, 54 bp, synthetic construct
  misc_feature 1..54: note = synthetic polynucleotide
  misc_feature 13..18: note = n = any nucleotide
  misc_feature 34..39: note = n = any nucleotide
  source 1..54: mol_type = other DNA
cgcagagtacgtnnnnnntagccatcgcattgcnnnnnntaccactgagctgaa

SEQ ID NO: 118 - DNA, 56 bp, synthetic construct
  misc_feature 1..56: note = synthetic polynucleotide
  misc_feature 25..32: note = n = any nucleotide
  misc_feature 36..41: note = n = any nucleotide
  source 1..56: mol_type = other DNA
baaaaaaaaaaaaaaaaaaaacgtnnnnnnnncgtnnnnnnttcagctcagtggta